European Patent Specification EP 2 954 046 B1, published October 15, 2025. Title: INDUCED PLURIPOTENT CELL-DERIVED OLIGODENDROCYTE PROGENITOR CELLS FOR THE TREATMENT OF MYELIN DISORDERS. Applicant: University of Rochester Goldman, Steven A. Wang, Su. The sequence listing filed with the application follows.

SEQUENCE LISTING (26 sequences)

SEQ ID NO: 1 - DNA, 21 bp, Artificial
  Primer
cgtctccacacatcagcacaa

SEQ ID NO: 2 - DNA, 22 bp, Artificial
  Primer
tcttggcagcaggatagtcctt

SEQ ID NO: 3 - DNA, 18 bp, Artificial
  Primer
ccacccatggcaaattcc

SEQ ID NO: 4 - DNA, 22 bp, Artificial
  Primer
tgggatttccattgatgacaag

SEQ ID NO: 5 - DNA, 20 bp, Artificial
  Primer
catcgagatcgccacctaca

SEQ ID NO: 6 - DNA, 19 bp, Artificial
  Primer
tctgcacgggaatggtgat

SEQ ID NO: 7 - DNA, 17 bp, Artificial
  Primer
tgcggccgattgtgaac

SEQ ID NO: 8 - DNA, 21 bp, Artificial
  Primer
cctcttttctctgcggaacgt

SEQ ID NO: 9 - DNA, 22 bp, Artificial
  Primer
accaggcactaccgtaaacaca

SEQ ID NO: 10 - DNA, 20 bp, Artificial
  Primer
ggtccgacctggaaaatgct

SEQ ID NO: 11 - DNA, 21 bp, Artificial
  Primer
ccaaaggcaaacaacccactt

SEQ ID NO: 12 - DNA, 20 bp, Artificial
  Primer
tcttgaccgggaccttgtct

SEQ ID NO: 13 - DNA, 17 bp, Artificial
  Primer
ggcgggcattccctttt

SEQ ID NO: 14 - DNA, 20 bp, Artificial
  Primer
cgagctgtactgggcgttgt

SEQ ID NO: 15 - DNA, 22 bp, Artificial
  Primer
tggtccgagtgtggttctgtaa

SEQ ID NO: 16 - DNA, 21 bp, Artificial
  Primer
tgtgcatagtcgctgcttgat

SEQ ID NO: 17 - DNA, 18 bp, Artificial
  Primer
ggcgcgcaactacatcct

SEQ ID NO: 18 - DNA, 19 bp, Artificial
  Primer
cgctcaccagtcgcttcat

SEQ ID NO: 19 - DNA, 19 bp, Artificial
  Primer
tcgggcaccacttcaacag

SEQ ID NO: 20 - DNA, 20 bp, Artificial
  Primer
tccgggaacttgaactggaa

SEQ ID NO: 21 - DNA, 19 bp, Artificial
  Primer
ccttggtggcaccccttac

SEQ ID NO: 22 - DNA, 22 bp, Artificial
  Primer
tccggtacccactcttgatctt

SEQ ID NO: 23 - DNA, 16 bp, Artificial
  Primer
tgcgagcgctgcacat

SEQ ID NO: 24 - DNA, 24 bp, Artificial
  Primer
gcagcgtgtacttatccttcttca

SEQ ID NO: 25 - DNA, 22 bp, Artificial
  Primer
ccacgaggtaatgtccaacatg

SEQ ID NO: 26 - DNA, 18 bp, Artificial
  Primer
cattgggcggcaggtact